European Patent Specification EP 3 674 404 B1, published October 15, 2025. Title: Target sequence-specific alteration technique using nucleotide target recognition. Applicant: Tokushima University. The sequence listing filed with the application follows.

SEQUENCE LISTING (45 sequences)

SEQ ID NO: 1 - protein, 224 aa, Microcystis aeruginosa
MVHIYSCQLELHDSLYYATREIGRLYESEPVIHNYALCYALGLVNSDSYRYFCSEQIPQYQEHLNPLNEEKIYVTPARAIAHTAVLNTWKYANNNYHVEMEKTQKNIPSFGRAKEIAPESIFECFIISHHPLQLPKWIRLGKWMSKAEVKLTELSLSKQKEDLFIYPYPLNPLDVMFTHQVIGYDVINMPPVSLIRNVRMRGEYYQISDRPDLKIPARLSYHFG

SEQ ID NO: 2 - protein, 277 aa, Microcystis aeruginosa
MPYSLVLNLTPRSPIYPNFLTGRHLHALFLTLVSSVDQELGNILHTAEADKAFTLSPLQMQSGGKTINSPQWRHEREIASETPCWWRISLLDDRLFGKLTSLWLNLNPKQPWHLGSADLVITSVLATPQSVQPWANSCTYQYLYENASETNREFDFLFATPVTFRQGKFDSALPTRELVFNSLLGRWNRYSGIPFDSIALESIFPSFFDIQTKLADEAYKNQSIGCVGEIHYRLLGEVEPAKIKAINALADFALYAGVGRKTTMGMGMTRRISKDKR

SEQ ID NO: 3 - protein, 332 aa, Microcystis aeruginosa
TFLTSVDAKFFHSEIPYKPMGKYVHFLTIRVTESYPLFQTDGELNKARVRAGIDSKKTISRLSMFKRKQSTPERLVGRELLRNYGLITAEECEYNVKFAMNNADCIIYGFAIGDSGSEKSKVVVDTAFSITPFDESHESFTLNAPYENGTMASKGENNTKVGEVTSRINQQDHIRPQVFFPSIVTLKDPTEASFLYVFNNILRTRHYGAQTTRTGRVRNELIGVIFADGEIVSNLRWTQAIYDRLPDEVLHSIDPLDEDLVMEKATEAIQALMAEEFIVHTDFIGENFQPLLTEVKTLTGTEAGILSVLDQANKESKKYFEQYIEKKKAEKK

SEQ ID NO: 4 - protein, 721 aa, Microcystis aeruginosa
MGNYQVTLKPVYSCPADEIPDGIKVPQGWRLSWHQVETWKALNDPDIDVIFNTAMTGDGKSLAAYLRTLQGYFPIMGLYPTNELARDQRGQIEAYIQRFQPTDQPRVNLLTGPELELYAERDGKTKAIALETRSKQSEILLTNPDIFHYLHRAAYLTPYDNPDQLWNRIDKHFDLFLFDEFHVFGTPQVASIINTMLLIRRANRGKRYLFLSATPDEGLLKRLDKAGFRYRSIDPVREGKYRFPDTPEEANSLAQQGWRQVTSEIELSFIPLPSSFQTSENWLKENKERILDYFKRYPGSKGAIILNSIASVKRLLPIFRELLATIGLTVGENTGLSGTREKLASLNRDLVIGTSTIDVGVDFKINFLIFESSDAGNFIQRFGRLGRHSGYDRKGTAVKFTNFTAIALVPKFFLERLFEKKDAPLQVGERYDRIQLQEAIKSNYRHINNFEGYYQRWGAVQSFQLWWNLGSPKIKSQYGESRQKFQQECEEVFDTSLKRVAGRVKGWADEWKELSGKNGNPIFEDASSFRGSSPLLCGLYDSTEPEECDRFKTYDLPSILGNLEVEVWRKGEFKRQIEATKTPIARRRFDYCLAFLNLKGYREERLNWRFTYDGDLGEIASAWKVQVLTGIGVWQPDNPWLDRISRELRDLALVSFVFAYPVAAVRQRLQLPMHFGIYPISDESSLHSPLSPYSIAIGQAALLLDTLAHRFKGKGGEVWIC

SEQ ID NO: 5 - protein, 1156 aa, Microcystis aeruginosa
MPKKQKKLEETGQLNLFDNTTEIDDEDLDFEFEDIDLESLVSEDLGITESVSDRRVETVRQLLTLKLLREAIRAENPDDRVMADFAEMVLPNLLRLAIGVTAKGGNFIEAVDRGRELRNKPKAKRDNAGDQSLNTHLLNGLFPANLIEKRLQKLNTTVRRIIKEFERRLAIAGFLVHDFEKFSYDRFPSMSERYIQIQRDFIQDPFKNQDPRKLSREEHREILQVLIPELGLDRFLFPDNPERWLEYLDDLLYIAKNTQRRNDTDLNTSEDGLNVRLNDRVIESLCDLACLADRLASIIKHPHDAEKASLQDLLYSLSDGELKFTYHSIAENRGVLTNVLNNAVMEAHQELDYQPLLYLPTGVVYIAPKNAPEVSLETLPNRVVDTIKSLCSGELQRKQTGFGRDGKGMKYADYYSQFFDDAGLMRAALNATLRILGDNKASVARSRGENLIKFQQQGVLPTDYDFHCEDDIRIDRLAEFGDVVTRKIWGDRLEKIEQARKLQKNLPAPPDLDLISEIAHYWNLENYLPQIRAIKRINESLKELKLKGNTGGVPYEWYYLAAQYLKQHPGIEDIRPVAEDLIAFLAAKIAAIVAGYNLPDGWEDLREWVNQVVQLPGRELAHSIETFQKELNHYNAAKKQGRGRQLLCSISHSPYSVSEQMESAVLFTPQVYTNKQMLAGSNAKRNISSIAGTEMMLRQILMNQTQAVGKRFEDGKYRYLYFYPTYYFTPETNSFLQKAYANIAQTRFDSSIKLHFVDKNLVANFDRTRYQSVDSFLIDEKLRQKKETINEEEDGKKDRTFKLSYPEDKPLTFYFMALPPGRNPTDTESWVMPAWLGLAFPMILDVKTVVSESPIPPYRDGAEFEETVFLDSAPQAIRSLTRCDRFRLDRVLNPWQDNDGKKYSAPLNTLTAAYSIHLDVNSKQGKTGYDPNWGKLTELAINLETSPLYVFHYFKQWKRGKDADIPSANRIALYLYDFYPCFDPYVQANRTNLTIDMTAESPLNHPKNLTELYRQFYRAKSSKGKPIKANAILKPIDEAADIILKADKAISDDLTSLVAARLFKLMDRVRSQTAEGRYVIKERDQEREKILDFAKYFVKNVFEESFESDRARLAGRQLNIIRDTCEFLYRLEMDKERRQRQVQPLDTSNSSSEEEE

SEQ ID NO: 6 - RNA, 109 nt, Artificial
  TiDcrRNA
  misc_feature (38)..(72): n is a, c, g, or u
guuccaauuaaucuuaagcccuauuagggauugaaacnnnnnnnnnnnnnnnnnnnnnnnnnnnnnnnnnnnguuccaauuaaucuuaagcccuauuagggauugaaac

SEQ ID NO: 7 - DNA, 675 bp, Artificial
  Cas5d nucleotide sequence for expression in Escherichia coli
atggtgcatatttatagctgccagctggaactgcatgatagcctgtattatgcgacccgcgaaattggccgcctgtatgaaagcgaaccggtgattcataactatgcgctgtgctatgcgctgggcctggtgaacagcgatagctatcgctatttctgcagcgaacagattccgcagtatcaggaacatctgaacccgctgaacgaagaaaaaatttatgtgaccccggcgcgcgcgattgcgcataccgcggtgctgaacacctggaaatatgcgaacaacaactatcatgtggaaatggaaaaaacccagaaaaacattccgagcttcggccgcgcgaaagaaattgcgccggaaagcattttcgaatgcttcattattagccatcatccgctgcagctgccgaaatggattcgcctgggcaaatggatgagcaaagcggaagtgaaactgaccgaactgagcctgagcaaacagaaagaagatctgttcatttatccgtatccgctgaacccgctggatgtgatgttcacccatcaggtgattggctatgatgtgattaacatgccgccggtgagcctgattcgcaacgtgcgcatgcgcggcgaatattatcagattagcgatcgcccggatctgaaaattccggcacgtctgagctatcatttcggctaa

SEQ ID NO: 8 - DNA, 834 bp, Artificial
  Cas6d nucleotide sequence for expression in Escherichia coli
atgccgtatagcctggtgctgaacctgaccccgcgcagcccgatttatccgaacttcctgaccggccgccatctgcatgcgctgttcctgaccctggtgagcagcgtggatcaggaactgggcaacattctgcataccgcggaagcggataaagcgttcaccctgagcccgctgcagatgcagagcggcggcaaaaccattaacagcccgcagtggcgccatgaacgcgaaattgcgagcgaaaccccgtgctggtggcgcattagcctgctggatgatcgcctgttcggcaaactgaccagcctgtggctgaacctgaacccgaaacagccgtggcatctgggcagcgcggatctggtgattaccagcgtgctggcgaccccgcagagcgtgcagccgtgggcgaacagctgcacctatcagtatctgtatgaaaacgcgagcgaaaccaaccgcgaattcgatttcctgttcgcgaccccggtgaccttccgccagggcaaattcgatagcgcgctgccgacccgcgaactggtgttcaacagcctgctgggccgctggaaccgctatagcggcattccgttcgatagcattgcgctggaaagcattttcccgagcttcttcgatattcagaccaaactggcggatgaagcgtataaaaaccagagcattggctgcgtgggcgaaattcattatcgcctgctgggcgaagtggaaccggcgaaaattaaagcgattaacgcgctggcggatttcgcgctgtatgcgggcgtgggccgcaaaaccaccatgggcatgggcatgacccgccgcattagcaaagataaacgctaa

SEQ ID NO: 9 - DNA, 1002 bp, Artificial
  Cas7d nucleotide sequence for expression in Escherichia coli
atgaccttcctgaccagcgtggatgcgaaattcttccatagcgaaattccgtataaaccgatgggcaaatatgtgcatttcctgaccattcgcgtgaccgaaagctatccgctgttccagaccgatggcgaactgaacaaagcgcgcgtgcgcgcgggcattgacagcaagaaaaccattagccgcctgagcatgttcaaacgcaaacagagcaccccggaacgcctggtgggccgcgaactgctgcgcaactatggcctgattaccgcggaagaatgcgaatataacgtgaaattcgcgatgaacaacgcggattgcattatttatggcttcgcgattggcgatagcggcagcgaaaaaagcaaagtggtggtggataccgcgttcagcattaccccgttcgatgaaagccatgagagcttcaccctgaacgcgccgtatgaaaacggcacgatggcgagcaaaggcgaaaacaacaccaaagtgggcgaagtgaccagccgcattaaccagcaggatcatattcgcccgcaggtgttcttcccgagcattgtgaccctgaaagatccgaccgaagcgagcttcctgtatgtgttcaacaacattctgcgcacccgccattatggcgcgcagaccacccgcaccggccgcgtgcgcaacgaactgattggcgtgattttcgcggatggcgaaattgtgagcaacctgcgctggacccaggcgatttatgatcgcctgccggatgaagtgctgcatagcattgatccgctggatgaagatctggtgatggaaaaagcgaccgaagcgattcaggcgctgatggcggaagaatttattgtgcataccgatttcattggcgaaaacttccagccgctgctgaccgaagtgaaaaccctgaccggcaccgaagcgggcattctgagcgtgctggatcaggcgaacaaagaaagcaaaaaatatttcgaacagtatattgaaaagaaaaaggcggaaaagaaataa

SEQ ID NO: 10 - DNA, 2166 bp, Artificial
  Cas3d nucleotide sequence for expression in Escherichia coli
atgggaaactatcaggtgactcttaagccagtgtattcttgcccagctgacgagatcccagacggaatcaaggtgccacagggatggagactttcttggcaccaggtggagacttggaaggctcttaacgacccagacatcgacgtgatcttcaacactgctatgactggagacggaaagtctcttgctgcttatcttagaactcttcagggatatttcccaatcatgggactttatccaactaacgagcttgctagagatcagagaggacagatcgaggcttatatccagagattccagccaactgaccagccaagagtgaaccttcttactggaccagagcttgagctttatgctgagagagacggaaagactaaggctatcgctcttgagactagatctaagcagtctgagatccttcttactaacccagacatcttccactatcttcacagagctgcttatcttactccatatgacaacccagaccagctttggaacagaatcgacaagcacttcgaccttttccttttcgacgagttccacgtgttcggaactccacaggtggcttctatcatcaacactatgcttcttatcagaagagctaacagaggaaagagatatcttttcctttctgctactccagacgagggacttcttaagagacttgacaaggctggattcagatatagatctatcgacccagtgagagagggaaagtatagattcccagacactccagaggaggctaactctcttgctcagcagggatggagacaggtgacttctgagatcgagctttctttcatcccacttccatcttctttccagacttctgagaactggcttaaggagaacaaggagagaatccttgactatttcaagagatatccaggatctaagggagctatcatccttaactctatcgcttctgtgaagagacttcttccaatcttcagagagcttcttgctactatcggacttactgtgggagagaacactggactttctggaactagagagaaacttgcttctcttaacagagatcttgtgatcggaacttctactatcgacgtgggagtggacttcaagatcaacttccttatcttcgagtcttctgacgctggaaacttcatccagagattcggaagacttggaagacactctggatatgacagaaagggaactgctgtgaagttcactaacttcactgctatcgctcttgtgccaaagttcttccttgagagacttttcgagaagaaggacgctccacttcaggtgggagagagatatgacagaatccagcttcaggaggctatcaagtctaactatagacacatcaacaacttcgagggatattatcagagatggggagctgtgcagtctttccagctttggtggaaccttggatctccaaagatcaagtctcagtatggagagtcaagacagaagttccagcaggagtgcgaggaggtgttcgacacttctcttaagagagtggctggaagagtgaagggatgggctgacgagtggaaggagctttctggaaagaacggaaacccaatcttcgaggacgcttcttctttcagaggatcttctccacttctttgcggactttatgactctactgagccagaggagtgcgacagattcaagacttatgaccttccatctatccttggaaaccttgaggtggaggtgtggagaaagggagagttcaagagacagatcgaggctactaagactccaatcgctagaagaagattcgactattgccttgctttccttaaccttaagggatatagagaggagagacttaactggagattcacttatgacggagatcttggagagatcgcttctgcttggaaggtgcaggtgcttactggaatcggagtgtggcagccagacaacccttggcttgacagaatctcaagagagcttagagatcttgctcttgtgtctttcgtgttcgcttatccagtggctgctgtgagacagagacttcagcttccaatgcacttcggaatctatccaatctctgacgagtcttctcttcactctccactttctccatattctatcgctatcggacaggctgctcttcttcttgacactcttgctcacagattcaagggaaagggaggagaggtgtggatctgctag

SEQ ID NO: 11 - DNA, 3471 bp, Artificial
  Cas10d nucleotide sequence for expression in Escherichia coli
atgccaaagaagcagaagaagcttgaggagactggacagcttaaccttttcgacaacactactgagatcgacgacgaggaccttgacttcgagttcgaggacatcgaccttgagtctcttgtgtctgaggaccttggaatcactgagtctgtgtctgacagaagagtggagactgtgagacagcttcttactcttaagcttcttagagaggctatcagagctgagaacccagacgacagagtgatggctgacttcgctgagatggtgcttccaaaccttcttagacttgctatcggagtgactgctaagggaggaaacttcatcgaggctgtggacagaggaagagagcttagaaacaagccaaaggctaagagagacaacgctggagatcagtctcttaacactcaccttcttaacggacttttcccagctaaccttatcgagaagagacttcagaagcttaacactactgtgagaagaatcatcaaggagttcgagagaagacttgctatcgctggattccttgtgcacgacttcgagaagttctcttatgacagattcccatctatgtctgagagatatatccagatccagagagacttcatccaggacccattcaagaaccaggacccaagaaagctttcaagagaggagcacagagagatccttcaggtgcttatcccagagcttggacttgacagattccttttcccagacaacccagagagatggcttgagtatcttgacgaccttctttatatcgctaagaacactcagagaagaaacgacactgaccttaacacttctgaggacggacttaacgtgagacttaacgacagagtgatcgagtctctttgcgaccttgcttgccttgctgacagacttgcttctatcatcaagcacccacacgacgctgagaaggcttctcttcaggaccttctttattctctttctgacggagagcttaagttcacttatcactctatcgctgagaacagaggagtgcttactaacgtgcttaacaacgctgtgatggaggctcaccaggagcttgactatcagccacttctttatcttccaactggagtggtgtatatcgctccaaagaacgctccagaggtgtctcttgagactcttccaaacagagtggtggacactatcaagtctctttgctctggagagcttcagagaaagcagactggattcggaagagacggaaagggtatgaagtatgctgactattattctcagttcttcgacgacgctggacttatgagagctgctcttaacgctactcttagaatccttggagacaacaaggcttctgtggctagatctagaggagagaaccttatcaagttccagcagcagggagtgcttccaactgactatgacttccactgcgaggacgacatcagaatcgacagacttgctgagttcggagacgtggtgactagaaagatctggggagacagacttgagaagatcgagcaggctagaaagcttcagaagaaccttccagctccaccagaccttgaccttatctctgagatcgctcactattggaaccttgagaactatcttccacagatcagagctatcaagagaatcaacgagtctcttaaggagcttaagcttaagggaaacactggaggagtgccatatgagtggtattatcttgctgctcagtatcttaagcagcacccaggaatcgaggacatcagaccagtggctgaggaccttatcgctttccttgctgctaagatcgctgctatcgtggctggatataaccttccagacggatgggaggaccttagagagtgggtgaaccaggtggtgcagcttccaggaagagagcttgctcactctatcgagactttccagaaggagcttaaccactataacgctgctaagaagcagggaagaggaagacagcttctttgctctatctctcactctccatattctgtgtctgagcagatggagtctgctgtgcttttcactccacaggtgtatactaacaagcagatgcttgctggatctaacgctaagagaaacatctcttctatcgctggaactgagatgatgcttagacagatccttatgaaccagactcaggctgtgggaaagagattcgaggacggaaagtatagatatctttatttctatccaacttattatttcactccagagactaactctttccttcagaaggcttatgctaacatcgctcagactagattcgactcttctatcaagcttcacttcgtggacaagaaccttgtggctaacttcgacagaactagatatcagtctgtggactctttccttatcgacgagaagcttagacagaagaaggagactatcaacgaggaggaggacggaaagaaggacagaactttcaagctttcttatccagaggacaagccacttactttctatttcatggctcttccaccaggaagaaacccaactgacactgagtcttgggtaatgccagcttggcttggacttgctttcccaatgatccttgacgtgaagactgtggtgtctgagtctccaatcccaccatatagagacggagctgagttcgaggagactgtgttccttgactctgctccacaggctatcagatctcttactagatgcgacagattcagacttgacagagtgcttaacccttggcaggacaacgacggaaagaagtattctgctccacttaacactcttactgctgcttattctatccaccttgacgtgaactctaagcagggaaagactggatatgacccaaactggggaaagcttactgagcttgctatcaaccttgagacttctccactttatgtgttccactatttcaagcagtggaagagaggaaaggacgctgacatcccatctgctaacagaatcgctctttatctttatgacttctatccatgcttcgacccatatgtgcaggctaacagaactaaccttactatcgacatgactgctgagtctccacttaaccacccaaagaaccttactgagctttatagacagttctatagagctaagtcttctaagggaaagccaatcaaggctaacgctatccttaagccaatcgacgaggctgctgacatcatccttaaggctgacaaggctatctctgacgaccttacttctcttgtggctgctagacttttcaagcttatggacagagtgagatctcagactgctgagggaagatatgtgatcaaggagagagatcaggagagagagaagatccttgacttcgctaagtatttcgtgaagaacgtgttcgaggagtctttcgagtctgacagagctagacttgctggaagacagcttaacatcatcagagacacttgcgagttcctttatagacttgagatggacaaggagagaagacagagacaggtgcagccacttgacacttctaactcttcttctgaggaggaggagtaa

SEQ ID NO: 12 - DNA, 35 bp, Artificial
  J23108 synthesis promoter
ctgacagctagctcagtcctaggtataatgctagc

SEQ ID NO: 13 - DNA, 36 bp, Artificial
  Ribosomal binding sequence
aataattttgtttaactttaagaaggagatatacat

SEQ ID NO: 14 - DNA, 24 bp, Artificial
  Terminator sequence STOP767
agatcctgtaaaacgacggccagt

SEQ ID NO: 15 - DNA, 19 bp, Artificial
  Terminator sequence STOP768(1)
cgccagggttttcccagtc

SEQ ID NO: 16 - DNA, 19 bp, Artificial
  Terminator sequence TOP768(2)
cgccagggttttcccagtc

SEQ ID NO: 17 - DNA, 47 bp, Artificial
  T7 terminator sequence
tagcataaccccttggggcctctaaacgggtcttgaggggttttttg

SEQ ID NO: 18 - DNA, 37 bp, Artificial
  CRISPR repeat sequence
gttccaattaatcttaagccctattagggattgaaac

SEQ ID NO: 19 - DNA, 19 bp, Artificial
  T7 promoter sequence
taatacgactcactatagg

SEQ ID NO: 20 - DNA, 109 bp, Artificial
  crRNA expression cassette
gttccaattaatcttaagccctattagggattgaaacggtaataatacgactcactatagggagaaaggatcgttccaattaatcttaagccctattagggattgaaac

SEQ ID NO: 21 - DNA, 581 bp, Artificial
  Synthesis cccdB gene expression cassette
aggctttaatacgactcactatagggagaaaggatccataaaggaggtaaataatgaagcagcgtattacagtgacagttgacagcgacagctatcagttgctcaaggcatatatgatgtcaatatctccggtctggtaagcacaaccatgcagaatgaagcccgtcgtctgcgtgccgaacgctggaaagcggaaaatcaggaagggatggctgaggtcgcccggtttattgaaatgaacggctcttttgctgacgagaacagggactggtgaaatgcagtttaaggtttacacctataaaagagagagccgttatcgtctgtttgtggatgtacagagtgatattattgacacgcccgggcgacggatggtgatccccctggccagtgcacgtctgctgtcagataaagtctcccgtgaactttacccggtggtgcatatcggggatgaaagctggcgcatgatgaccaccgatatggccagtgtgccggtctccgttatcggggaagaagtggctgatctcagccaccgcgaaaatgacatcaaaaacgccattaacctgatgttctggggaatataa

SEQ ID NO: 22 - protein, 18 aa, Artificial
  Nuclear localizing signal (NLS) amino acid sequence
DPKKKRKVDPKKKRKVSG

SEQ ID NO: 23 - DNA, 54 bp, Artificial
  NLS nucleotide sequence
gacccaaagaagaagcggaaggtagaccctaagaagaagcgcaaggtttctgga

SEQ ID NO: 24 - protein, 20 aa, Artificial
  Self-cleaving peptide 2A amino acid sequence
GSEGRGSLLTCGDVEENPGP

SEQ ID NO: 25 - DNA, 60 bp, Artificial
  Self-cleaving peptide 2A(1) coding sequence
ggctctgagggcagaggcagcctgctgacctgcggcgacgtggaggaaaaccctggccct

SEQ ID NO: 26 - DNA, 60 bp, Artificial
  Self-cleaving peptide 2A(2) coding sequence
gggtctgagggacgcggctccctgctcacctgtggagatgtggaagagaacccaggcccc

SEQ ID NO: 27 - DNA, 60 bp, Artificial
  Self-cleaving peptide 2A(3) coding sequence
ggttctgaaggcagaggctctctgctgacatgtggggatgtggaggaaaatcctggccct

SEQ ID NO: 28 - DNA, 60 bp, Artificial
  Self-cleaving peptide 2A(4) coding sequence
ggatccgagggcagaggaagtctgctaacatgcggtgacgttgaggagaatcccgggcca

SEQ ID NO: 29 - DNA, 820 bp, Artificial
  2 x cauliflower mosaic virus 35S gene promoter + omega sequence
gccaacatggtggagcacgacactctcgtctactccaagaatatcaaagatacagtctcagaagaccaaagggctattgagacttttcaacaaagggtaatatcgggaaacctcctcggattccattgcccagctatctgtcacttcatcaaaaggacagtagaaaaggaaggtggcacctacaaatgccatcattgcgataaaggaaaggctatcgttcaagatgcctctgccgacagtggtcccaaagatggacccccacccacgaggagcatcgtggaaaaagaagacgttccaaccacgtcttcaaagcaagtggattgatgtgaacatggtggagcacgacactctcgtctactccaagaatatcaaagatacagtctcagaagaccaaagggctattgagacttttcaacaaagggtaatatcgggaaacctcctcggattccattgcccagctatctgtcacttcatcaaaaggacagtagaaaaggaaggtggcacctacaaatgccatcattgcgataaaggaaaggctatcgttcaagatgcctctgccgacagtggtcccaaagatggacccccacccacgaggagcatcgtggaaaaagaagacgttccaaccacgtcttcaaagcaagtggattgatgtgatatctccactgacgtaagggatgacgcacaatcccactatccttcgcaagacccttcctctatataaggaagttcatttcatttggagaggccggtctagagtatttttacaacaattaccaacaacaacaaacaacaaacaacattacaattactatttacaatt

SEQ ID NO: 30 - DNA, 447 bp, Artificial
  Arabidopsis shock protein 18.2kDa gene terminator
atatgaagatgaagatgaaatatttggtgtgtcaaataaaaagcttgtgtgcttaagtttgtgtttttttcttggcttgttgtgttatgaatttgtggctttttctaatattaaatgaatgtaagatctcattataatgaataaacaaatgtttctataatccattgtgaatgttttgttggatctcttctgcagcatataactactgtatgtgctatggtatggactatggaatatgattaaagataagatgggctcatagagtaaaacgaggcgagggacctataaacctcccttcatcatgctatttcatgatctattttataaaataaagatgtagaaaaaagtaagcgtaataaccgcaaaacaaatgatttaaaacatggcacataatgaggagattaagttcggtttacgtttattttagtactaattgtaacgtgagac

SEQ ID NO: 31 - DNA, 97 bp, Artificial
  crRNA expression cassette
gttccaattaatcttaagccctattagggattgaaacggagaccctcaattgtcggtctcgttccaattaatcttaagccctattagggattgaaac

SEQ ID NO: 32 - DNA, 448 bp, Artificial
  Arabidopsis U6 snRNA-26 gene promoter sequence
aagcttcgttgaacaacggaaactcgacttgccttccgcacaatacatcatttcttcttagctttttttcttcttcttcgttcatacagtttttttttgtttatcagcttacattttcttgaaccgtagctttcgttttcttctttttaactttccattcggagtttttgtatcttgtttcatagtttgtcccaggattagaatgattaggcatcgaaccttcaagaatttgattgaataaaacatcttcattcttaagatatgaagataatcttcaaaaggcccctgggaatctgaaagaagagaagcaggcccatttatatgggaaagaacaatagtatttcttatataggcccatttaagttgaaaacaatcttcaaaagtcccacatcgcttagataagaaaacgaagctgagtttatatacagctagagtcgaagtagtgatt

SEQ ID NO: 33 - DNA, 723 bp, Artificial
  2xNLS + Cas5d
gacccaaagaagaagcggaaggtagaccctaagaagaagcgcaaggtttctggagtgcacatctattcttgccagcttgagcttcacgactctctttattatgctactagagagatcggaagactttatgagtctgagccagtgatccacaactatgctctttgctatgctcttggacttgtgaactctgactcttatagatatttctgctctgagcagatcccacagtatcaggagcaccttaacccacttaacgaggagaagatctatgtgactccagctagagctatcgctcacactgctgtgcttaacacttggaagtatgctaacaacaactatcacgtggagatggagaagactcagaagaacatcccatctttcggaagagctaaggagatcgctccagagtctatcttcgagtgcttcatcatctctcaccacccacttcagcttccaaagtggatcagacttggaaagtggatgtctaaggctgaggtgaagcttactgagctttctctttctaagcagaaggaggaccttttcatctatccatatccacttaacccacttgacgtgatgttcactcaccaggttatcggatatgacgtgatcaacatgccaccagtgtctcttatcagaaacgtgagaatgagaggagagtattatcagatctctgacagaccagaccttaagatcccagctagactttcttatcacttcgga

SEQ ID NO: 34 - DNA, 882 bp, Artificial
  2xNLS + Cas6d
gacccaaagaagaagcggaaggtagaccctaagaagaagcgcaaggtttctggaccatattctcttgtgcttaaccttactccaagatctccaatctatccaaacttccttactggaagacaccttcacgctcttttccttactcttgtgtcttctgtggaccaggagcttggaaacatccttcacactgctgaggctgacaaggctttcactctttctccacttcagatgcagtctggaggaaagactatcaactctccacagtggagacacgagagagagatcgcttctgagactccatgctggtggagaatctctcttcttgacgacagacttttcggaaagcttacttctctttggcttaaccttaacccaaagcagccttggcaccttggatctgctgaccttgtgatcacttctgtgcttgctactccacagtctgtgcagccttgggctaactcttgcacttatcagtatctttatgagaacgcttctgagactaacagagagttcgacttccttttcgctactccagtgactttcagacagggaaagttcgactctgctcttccaactagagagcttgtgttcaactctcttcttggaagatggaacagatattctggaatcccattcgactctatcgctcttgagtctatcttcccatctttcttcgacatccagactaagcttgctgacgaggcttataagaaccagtctatcggatgcgtgggagagatccactatagacttcttggagaggtggagccagctaagatcaaggctatcaacgctcttgctgacttcgctctttatgctggagtgggaagaaagactactatgggaatgggaatgactagaagaatctctaaggacaagaga

SEQ ID NO: 35 - DNA, 1053 bp, Artificial
  2xNLS + Cas7d
gacccaaagaagaagcggaaggtagaccctaagaagaagcgcaaggtttctggaactttccttacttctgtggacgctaagttcttccactctgagatcccatataagccaatgggaaagtatgtgcacttccttactatcagagtgactgagtcttatccacttttccagactgacggagagcttaacaaggctagagtgagagctggaatcgactctaagaagactatctcaagactttctatgttcaagagaaagcagtctactccagagagacttgtgggaagagagcttcttagaaactatggacttatcactgctgaggagtgcgagtataacgtgaagttcgctatgaacaacgctgactgcatcatctatggattcgctatcggagactctggatctgagaagtctaaggtggtggtggacactgctttctctatcactccattcgacgagtctcacgagtctttcactcttaacgctccatatgagaacggaactatggcttctaagggagagaacaacactaaggtgggagaggtgacttcaagaatcaaccagcaggaccacatcagaccacaggtgttcttcccatctatcgtgactcttaaggacccaactgaggcttctttcctttatgtgttcaacaacatccttagaactagacactatggtgctcagactactagaactggaagagtgagaaacgagcttatcggagtgatcttcgctgacggagagatcgtgtctaaccttagatggactcaggctatctatgacagacttccagacgaggtgcttcactctatcgacccacttgacgaggaccttgtgatggagaaggctactgaggctatccaggctcttatggctgaggagttcatcgtgcacactgacttcatcggagagaacttccagccacttcttactgaggtgaagactcttactggaactgaggctggaatcctttctgtgcttgaccaggctaacaaggagtctaagaagtatttcgagcagtatatcgagaagaagaaggctgagaagaagtaa

SEQ ID NO: 36 - DNA, 2217 bp, Artificial
  2xNLS + Cas3d
atggacccaaagaagaagcggaaggtagaccctaagaagaagcgcaaggtttctggaggaaactatcaggtgactcttaagccagtgtattcttgcccagctgacgagatcccagacggaatcaaggtgccacagggatggagactttcttggcaccaggtggagacttggaaggctcttaacgacccagacatcgacgtgatcttcaacactgctatgactggagacggaaagtctcttgctgcttatcttagaactcttcagggatatttcccaatcatgggactttatccaactaacgagcttgctagagatcagagaggacagatcgaggcttatatccagagattccagccaactgaccagccaagagtgaaccttcttactggaccagagcttgagctttatgctgagagagacggaaagactaaggctatcgctcttgagactagatctaagcagtctgagatccttcttactaacccagacatcttccactatcttcacagagctgcttatcttactccatatgacaacccagaccagctttggaacagaatcgacaagcacttcgaccttttccttttcgacgagttccacgtgttcggaactccacaggtggcttctatcatcaacactatgcttcttatcagaagagctaacagaggaaagagatatcttttcctttctgctactccagacgagggacttcttaagagacttgacaaggctggattcagatatagatctatcgacccagtgagagagggaaagtatagattcccagacactccagaggaggctaactctcttgctcagcagggatggagacaggtgacttctgagatcgagctttctttcatcccacttccatcttctttccagacttctgagaactggcttaaggagaacaaggagagaatccttgactatttcaagagatatccaggatctaagggagctatcatccttaactctatcgcttctgtgaagagacttcttccaatcttcagagagcttcttgctactatcggacttactgtgggagagaacactggactttctggaactagagagaaacttgcttctcttaacagagatcttgtgatcggaacttctactatcgacgtgggagtggacttcaagatcaacttccttatcttcgagtcttctgacgctggaaacttcatccagagattcggaagacttggaagacactctggatatgacagaaagggaactgctgtgaagttcactaacttcactgctatcgctcttgtgccaaagttcttccttgagagacttttcgagaagaaggacgctccacttcaggtgggagagagatatgacagaatccagcttcaggaggctatcaagtctaactatagacacatcaacaacttcgagggatattatcagagatggggagctgtgcagtctttccagctttggtggaaccttggatctccaaagatcaagtctcagtatggagagtcaagacagaagttccagcaggagtgcgaggaggtgttcgacacttctcttaagagagtggctggaagagtgaagggatgggctgacgagtggaaggagctttctggaaagaacggaaacccaatcttcgaggacgcttcttctttcagaggatcttctccacttctttgcggactttatgactctactgagccagaggagtgcgacagattcaagacttatgaccttccatctatccttggaaaccttgaggtggaggtgtggagaaagggagagttcaagagacagatcgaggctactaagactccaatcgctagaagaagattcgactattgccttgctttccttaaccttaagggatatagagaggagagacttaactggagattcacttatgacggagatcttggagagatcgcttctgcttggaaggtgcaggtgcttactggaatcggagtgtggcagccagacaacccttggcttgacagaatctcaagagagcttagagatcttgctcttgtgtctttcgtgttcgcttatccagtggctgctgtgagacagagacttcagcttccaatgcacttcggaatctatccaatctctgacgagtcttctcttcactctccactttctccatattctatcgctatcggacaggctgctcttcttcttgacactcttgctcacagattcaagggaaagggaggagaggtgtggatctgc

SEQ ID NO: 37 - DNA, 3519 bp, Artificial
  2xNLS + Cas10d
gacccaaagaagaagcggaaggtagaccctaagaagaagcgcaaggtttctggaccaaagaagcagaagaagcttgaggagactggacagcttaaccttttcgacaacactactgagatcgacgacgaggaccttgacttcgagttcgaggacatcgaccttgagtctcttgtgtctgaggaccttggaatcactgagtctgtgtctgacagaagagtggagactgtgagacagcttcttactcttaagcttcttagagaggctatcagagctgagaacccagacgacagagtgatggctgacttcgctgagatggtgcttccaaaccttcttagacttgctatcggagtgactgctaagggaggaaacttcatcgaggctgtggacagaggaagagagcttagaaacaagccaaaggctaagagagacaacgctggagatcagtctcttaacactcaccttcttaacggacttttcccagctaaccttatcgagaagagacttcagaagcttaacactactgtgagaagaatcatcaaggagttcgagagaagacttgctatcgctggattccttgtgcacgacttcgagaagttctcttatgacagattcccatctatgtctgagagatatatccagatccagagagacttcatccaggacccattcaagaaccaggacccaagaaagctttcaagagaggagcacagagagatccttcaggtgcttatcccagagcttggacttgacagattccttttcccagacaacccagagagatggcttgagtatcttgacgaccttctttatatcgctaagaacactcagagaagaaacgacactgaccttaacacttctgaggacggacttaacgtgagacttaacgacagagtgatcgagtctctttgcgaccttgcttgccttgctgacagacttgcttctatcatcaagcacccacacgacgctgagaaggcttctcttcaggaccttctttattctctttctgacggagagcttaagttcacttatcactctatcgctgagaacagaggagtgcttactaacgtgcttaacaacgctgtgatggaggctcaccaggagcttgactatcagccacttctttatcttccaactggagtggtgtatatcgctccaaagaacgctccagaggtgtctcttgagactcttccaaacagagtggtggacactatcaagtctctttgctctggagagcttcagagaaagcagactggattcggaagagacggaaagggtatgaagtatgctgactattattctcagttcttcgacgacgctggacttatgagagctgctcttaacgctactcttagaatccttggagacaacaaggcttctgtggctagatctagaggagagaaccttatcaagttccagcagcagggagtgcttccaactgactatgacttccactgcgaggacgacatcagaatcgacagacttgctgagttcggagacgtggtgactagaaagatctggggagacagacttgagaagatcgagcaggctagaaagcttcagaagaaccttccagctccaccagaccttgaccttatctctgagatcgctcactattggaaccttgagaactatcttccacagatcagagctatcaagagaatcaacgagtctcttaaggagcttaagcttaagggaaacactggaggagtgccatatgagtggtattatcttgctgctcagtatcttaagcagcacccaggaatcgaggacatcagaccagtggctgaggaccttatcgctttccttgctgctaagatcgctgctatcgtggctggatataaccttccagacggatgggaggaccttagagagtgggtgaaccaggtggtgcagcttccaggaagagagcttgctcactctatcgagactttccagaaggagcttaaccactataacgctgctaagaagcagggaagaggaagacagcttctttgctctatctctcactctccatattctgtgtctgagcagatggagtctgctgtgcttttcactccacaggtgtatactaacaagcagatgcttgctggatctaacgctaagagaaacatctcttctatcgctggaactgagatgatgcttagacagatccttatgaaccagactcaggctgtgggaaagagattcgaggacggaaagtatagatatctttatttctatccaacttattatttcactccagagactaactctttccttcagaaggcttatgctaacatcgctcagactagattcgactcttctatcaagcttcacttcgtggacaagaaccttgtggctaacttcgacagaactagatatcagtctgtggactctttccttatcgacgagaagcttagacagaagaaggagactatcaacgaggaggaggacggaaagaaggacagaactttcaagctttcttatccagaggacaagccacttactttctatttcatggctcttccaccaggaagaaacccaactgacactgagtcttgggtaatgccagcttggcttggacttgctttcccaatgatccttgacgtgaagactgtggtgtctgagtctccaatcccaccatatagagacggagctgagttcgaggagactgtgttccttgactctgctccacaggctatcagatctcttactagatgcgacagattcagacttgacagagtgcttaacccttggcaggacaacgacggaaagaagtattctgctccacttaacactcttactgctgcttattctatccaccttgacgtgaactctaagcagggaaagactggatatgacccaaactggggaaagcttactgagcttgctatcaaccttgagacttctccactttatgtgttccactatttcaagcagtggaagagaggaaaggacgctgacatcccatctgctaacagaatcgctctttatctttatgacttctatccatgcttcgacccatatgtgcaggctaacagaactaaccttactatcgacatgactgctgagtctccacttaaccacccaaagaaccttactgagctttatagacagttctatagagctaagtcttctaagggaaagccaatcaaggctaacgctatccttaagccaatcgacgaggctgctgacatcatccttaaggctgacaaggctatctctgacgaccttacttctcttgtggctgctagacttttcaagcttatggacagagtgagatctcagactgctgagggaagatatgtgatcaaggagagagatcaggagagagagaagatccttgacttcgctaagtatttcgtgaagaacgtgttcgaggagtctttcgagtctgacagagctagacttgctggaagacagcttaacatcatcagagacacttgcgagttcctttatagacttgagatggacaaggagagaagacagagacaggtgcagccacttgacacttctaactcttcttctgaggaggaggag

SEQ ID NO: 38 - DNA, 35 bp, Nicotiana benthamiana
tgggtggtttgtctacagcaaaatatctggcagat

SEQ ID NO: 39 - DNA, 35 bp, Nicotiana benthamiana
aaatttgctattggactcttgccagcaatgcttgg

SEQ ID NO: 40 - DNA, 35 bp, Solanum lycopersicum
tacctggatctcagtctcccgaaagaggtgaggag

SEQ ID NO: 41 - DNA, 811 bp, Artificial
  Cytomegalovirus enhancer + universal chicken beta-actin gene hybrid promoter
cgttacataacttacggtaaatggcccgcctggctgaccgcccaacgacccccgcccattgacgtcaatagtaacgccaatagggactttccattgacgtcaatgggtggagtatttacggtaaactgcccacttggcagtacatcaagtgtatcatatgccaagtacgccccctattgacgtcaatgacggtaaatggcccgcctggcattgtgcccagtacatgaccttatgggactttcctacttggcagtacatctacgtattagtcatcgctattaccatggtcgaggtgagccccacgttctgcttcactctccccatctcccccccctccccacccccaattttgtatttatttattttttaattattttgtgcagcgatgggggcggggggggggggggggcgcgcgccaggcggggcggggcggggcgaggggcggggcggggcgaggcggagaggtgcggcggcagccaatcagagcggcgcgctccgaaagtttccttttatggcgaggcggcggcggcggcggccctataaaaagcgaagcgcgcggcgggcgggagtcgctgcgacgctgccttcgccccgtgccccgctccgccgccgcctcgcgccgcccgccccggctctgactgaccgcgttactcccacaggtgagcgggcgggacggcccttctcctccgggctgtaattagctgagcaagaggtaagggtttaagggatggttggttggtggggtattaatgtttaattacctggagcacctgcctgaaatcactttttttcaggttggaccggtgccacc

SEQ ID NO: 42 - DNA, 223 bp, Artificial
  Bovine-derived growth hormone gene terminator sequence
gctgatcagcctcgactgtgccttctagttgccagccatctgttgtttgcccctcccccgtgccttccttgaccctggaaggtgccactcccactgtcctttcctaataaaatgaggaaattgcatcgcattgtctgagtaggtgtcattctattctggggggtggggtggggcaggacagcaagggggaggattgggaagagaatagcaggcatgctgggga

SEQ ID NO: 43 - DNA, 249 bp, Artificial
  Human U6 snRNA gene promoter
gagggcctatttcccatgattccttcatatttgcatatacgatacaaggctgttagagagataattggaattaatttgactgtaaacacaaagatattagtacaaaatacgtgacgtagaaagtaataatttcttgggtagtttgcagttttaaaattatgttttaaaatggactatcatatgcttaccgtaacttgaaagtatttcgatttcttggctttatatatcttgtggaaaggacgaaacacc

SEQ ID NO: 44 - DNA, 35 bp, Homo sapiens
ccagaaccggaggacaaagtacaaacggcagaagc

SEQ ID NO: 45 - DNA, 35 bp, Homo sapiens
gatgtgatgggagcccttcttcttctgctcggact